European Patent Application EP 4 578 946 A1, published July 2, 2025. Title: OPTIMIZED GUIDE RNA, CRISPR/ACC2C9 GENE EDITING SYSTEM, AND GENE EDITING METHOD. Applicant: ShanghaiTech University. The sequence listing filed with the application follows.

SEQUENCE LISTING (140 sequences)

SEQ ID NO: 1 - protein, 506 aa, synthetic construct
MVQTEILKAFRFALDPTSVQVAALSRHAGAARWAFNHALAAKVGAHERWRAEVAKLVGDGVPEEQARRQVRVPVPMKPAIQKALNAVKGDSRKGLDGACPWWHEVNTYAFQSAFIDADQAWKNWLDSLSGKRVGRRVGYPRFKKKGRARDSFRLHHDVKKPSIRLAGYRRLRLPRIGEVRLHDSGKRLARLIDRGDAVVQSVTVSRGGHRWYASVLCKVTVQVPDRPSRRQRERGAVGVDLGVKVLAALSKPLVVDDPSSALVRNPQHLRQAERRLLKAQRALARTQKGSARREKAKRRVGRAHHEVAVRRHAALHQITKRLTTGFAVVALEDLNVAGMTRSARGTVAAPGKNVRQKAGLNRVILDSAPAELRRQVNYKATWYGSELAVADRWFPSSKTCSGCGWQNPHLKLSDRVFRCTDCGLVMDRAMNAARNIERHAVLIDRNVACDRRETLNARGASIRPTTSRGGRHDASKREGSGARPESPQQSDLLTLPTLNNETATPP

SEQ ID NO: 2 - DNA, 1521 bp, synthetic construct
  source 1..1521: mol_type = other DNA
atggtgcagacggagatcctgaaggcgtttcggtttgcgttggatccgacgtctgtgcaggttgctgccctttcccggcatgctggtgcggccaggtgggcgttcaaccatgctctcgcggccaaggtcggcgcgcatgagcggtggcgggcggaggtagccaagcttgtcggggacggtgttcctgaggagcaggctcgtaggcaggtgcgcgtcccggttccgatgaagccggcgatccagaaggcgttgaacgcggtcaagggtgactctcgcaagggcttggatggtgcgtgcccgtggtggcatgaggtcaacacttacgcgttccagtccgctttcatcgacgcggaccaggcgtggaagaactggttggactcgttgtcggggaagcgggtcggccgccgggtggggtacccgcggttcaagaagaaggggcgggcccgcgactcgtttcgcttgcaccacgacgtgaagaagccaagcatccggctggccgggtaccggcggttgcggctgccgaggatcggggaagtccggcttcatgactcggggaagcgtctggcacggctgatcgaccgaggtgacgcggtggtgcagtcggtgacggtgtcgcggggtggccatcgctggtatgcgtctgtgctgtgcaaggtcaccgtgcaggtaccggatcggccgtcacggcgccagcgggaacgaggcgctgttggggtggaccttggcgttaaggtcctcgcggctttgtccaagccactggtggtcgacgacccgtcgagtgccctggtgcggaatccgcagcatctgcggcaggccgagcggcgtctactgaaggctcagcgggcgttggcgcgtacacaaaaaggttcagcccgacgcgagaaggccaagcggcgagttggtcgcgcgcatcacgaggttgctgtgcgccggcatgctgcgctccatcagatcaccaagcgcctgaccaccggcttcgcggtcgtcgcgcttgaggatctgaacgtggccggtatgacaaggtcagcgcggggaacagtggcagcgccgggaaagaacgtgcggcagaaggcaggcctgaaccgcgtcatcctggactccgctccagccgagttgcgtcgccaggtgaactacaaggccacctggtatggatctgagctggcggtcgcagaccgctggttcccctcgagtaagacctgttcgggttgcggatggcaaaacccacacctgaagctgtccgacagggtgtttcgttgcacagactgcgggctggtgatggaccgggccatgaacgcggcccggaacatcgaacgccacgcagtgctgatcgatcgaaacgtcgcctgcgataggcgggagacgctaaacgcccgtggagcatccataagaccaaccacctctcggggcggtaggcacgacgcatcgaagcgggaaggctccggcgctcggcctgagtcacctcagcagagtgatctgctgacgctcccaaccttgaataacgaaacggcaacgcctccataa

SEQ ID NO: 3 - DNA, 1518 bp, synthetic construct
  source 1..1518: mol_type = other DNA
atggtgcagacagagatcctgaaggcctttcggttcgccctcgatcctacttccgtccaggtggccgccctgagccggcacgccggggccgccaggtgggccttcaaccacgccctcgccgccaaggtgggggcccacgagcggtggcgggccgaggtggccaagctcgtgggcgatggcgtgcccgaggagcaggcccggcggcaggtccgggtccccgtgcctatgaagccagccatccagaaggccctgaacgccgtgaagggggattcccggaagggcctggatggggcctgcccatggtggcacgaggtgaacacctacgccttccagagcgcctttattgacgccgaccaggcatggaagaactggctcgacagcctgagcggcaagagagtggggaggagggtgggctacccccggtttaagaagaagggccgggctcgggatagctttagattgcaccacgatgtgaagaagcccagcatcaggctggctggctacagaaggctgaggctgcctaggattggcgaggtgaggctgcacgacagcggcaagcggctcgccaggctcattgacagaggcgacgccgtggtgcagtccgtgactgtgagtaggggcggacacaggtggtacgcctccgtgctctgcaaggtgacagtgcaggtgcccgatcggcccagcaggcggcagcgggagaggggcgccgtgggagtggacctgggggtgaaggtgctggccgccctgtccaagcccctggtcgtcgacgacccaagcagcgccctggtgagaaacccccagcacctgaggcaggctgagaggcggctgctcaaggcccagcgggccctggccaggacacagaagggcagcgccaggagagagaaggccaagcggcgggtggggagggcccatcacgaggtggccgtccggcggcacgccgccctgcaccagatcaccaagcggctgaccacagggttcgccgtggtggccctggaggatctgaacgtcgccggcatgaccaggtccgccagggggacagtggccgccccagggaagaacgtccggcagaaggccgggctgaaccgggtcatcctggacagcgcccctgccgagctgcggaggcaggtgaactacaaggccacctggtacgggagcgagctggccgtggccgacaggtggttcccctccagcaagacctgcagcgggtgcggctggcagaacccccacttgaagctctccgatagggtgtttaggtgcaccgactgcggcctggtcatggatagagatatgaacgccgctaggaacatcgagaggcacgctgtgttgattgataggaacgtggcctgcgaccggcgggagactttgaacgccaggggggccagcatccggcccaccacaagccggggggggcggcacgacgccagcaagagggaggggagcggggcccggccagagtccccccagcagtctgatctgctcacactccccacactgaacaacgaaaccgccacacccccc

SEQ ID NO: 4 - RNA, 299 nt, synthetic construct
  source 1..299: mol_type = other RNA
gaacgcggcccggaacatcgaacgccacgcagtgctgatcgatcgaaacgtcgcctgcgataggcgggagacgctaaacgcccgtggagcatccataagaccaaccacctctcggggcggtaggcacgacgcatcgaagcgggaaggctccggcgctcggcctgagtcacctcagcagagtgatctgctgacgctcccaaccttgaataacgaaacggcaacgcctccatagcggtgcaggtcaataagggtcggccccacgcgtgtagggagcgatcgagtgacagtatcctctgtat

SEQ ID NO: 5 - RNA, 270 nt, synthetic construct
  source 1..270: mol_type = other RNA
cagtgctgatcgatcgaaacgtcgcctgcgataggcgggagacgctaaacgcccgtggagcatccataagaccaaccacctctcggggcggtaggcacgacgcatcgaagcgggaaggctccggcgctcggcctgagtcacctcagcagagtgatctgctgacgctcccaaccttgaataacgaaacggcaacgcctccatagcggtgcaggtcaataagggtcggccccacgcgtgtagggagcgatcgagtgacagtatcctctgtat

SEQ ID NO: 6 - RNA, 240 nt, synthetic construct
  source 1..240: mol_type = other RNA
cagtgctgatcgatcgaaacgtcgcctgcgataggcgggagacgctaaacgcccgtggagcatccataagaccaaccacctctcggggcggtaggcacgacgcatcgaagcgggaaggctccggcgctcggcctgagtcacctcagcagagtgatctgctgacgctcccaaccttgaataacgaaacgaaagtcggccccacgcgtgtagggagcgatcgagtgacagtatcctctgtat

SEQ ID NO: 7 - RNA, 231 nt, synthetic construct
  source 1..231: mol_type = other RNA
cagtgctgatcgatcgaaacgtcgcctgcgataggcgggagacgctaaacgcccgtggagcatccataagaccaaccacctctcggggcggtaggcacgacgcatcgaagcgggaaggctccggcgctcggcctgagtcacctcagcagagtgatctgctgacgctcccaaccttgaataacggaaaccccacgcgtgtagggagcgatcgagtgacagtatcctctgtat

SEQ ID NO: 8 - RNA, 223 nt, synthetic construct
  source 1..223: mol_type = other RNA
cagtgctgatcgatcgaaacgtcgcctgcgataggcgggagacgctaaacgcccgtggagcatccataagaccaaccacctctcggggcggtaggcacgacgcatcgaagcgggaaggctccggcgctcggcctgagtcacctcagcagagtgatctgctgacgctcccaaccttgaatgaaaacgcgtgtagggagcgatcgagtgacagtatcctctgtat

SEQ ID NO: 9 - RNA, 217 nt, synthetic construct
  source 1..217: mol_type = other RNA
cagtgctgatcgatcgaaacgtcgcctgcgataggcgggagacgctaaacgcccgtggagcatccataagaccaaccacctctcggggcggtaggcacgacgcatcgaagcgggaaggctccggcgctcggcctgagtcacctcagcagagtgatctgctgacgctcccaaccttggaaacgtgtagggagcgatcgagtgacagtatcctctgtat

SEQ ID NO: 10 - RNA, 210 nt, synthetic construct
  source 1..210: mol_type = other RNA
cagtgctgatcgatcgaaacgtcgcctgcgataggcgggagacgctaaacgcccgtggagcatccataagaccaaccacctctcggggcggtaggcacgacgcatcgaagcgggaaggctccggcgctcggcctgagtcacctcagcagagtgatctgctgacgctcccaacgaaagtagggagcgatcgagtgacagtatcctctgtat

SEQ ID NO: 11 - RNA, 204 nt, synthetic construct
  source 1..204: mol_type = other RNA
cagtgctgatcgatcgaaacgtcgcctgcgataggcgggagacgctaaacgcccgtggagcatccataagaccaaccacctctcggggcggtaggcacgacgcatcgaagcgggaaggctccggcgctcggcctgagtcacctcagcagagtgatctgctgacgctcccgaaagggagcgatcgagtgacagtatcctctgtat

SEQ ID NO: 12 - RNA, 200 nt, synthetic construct
  source 1..200: mol_type = other RNA
cagtgctgatcgatcgaaacgtcgcctgcgataggcgggagacgctaaacgcccgtggagcatccataagaccaaccacctctcggggcggtaggcacgacgcatcgaagcgggaaggctccggcgctcggcctgagtcacctcagcagagtgatctgctgacgctcgaaagagcgatcgagtgacagtatcctctgtat

SEQ ID NO: 13 - RNA, 196 nt, synthetic construct
  source 1..196: mol_type = other RNA
cagtgctgatcgatcgaaacgtcgcctgcgataggcgggagacgctaaacgcccgtggagcatccataagaccaaccacctctcggggcggtaggcacgacgcatcgaagcgggaaggctccggcgctcggcctgagtcacctcagcagagtgatctgctgacgcgaaagcgatcgagtgacagtatcctctgtat

SEQ ID NO: 14 - RNA, 192 nt, synthetic construct
  source 1..192: mol_type = other RNA
cagtgctgatcgatcgaaacgtcgcctgcgataggcgggagacgctaaacgcccgtggagcatccataagaccaaccacctctcggggcggtaggcacgacgcatcgaagcgggaaggctccggcgctcggcctgagtcacctcagcagagtgatctgctgacgaaagatcgagtgacagtatcctctgtat

SEQ ID NO: 15 - RNA, 310 nt, synthetic construct
  source 1..310: mol_type = other RNA
gaacgcggcccggaacatcgaacgccacgcagtgctgatcgatcgaaacgtcgcctgcgataggcgggagacgctaaacgcccgtggagcatccataagaccaaccacctctcggggcggtaggcacgacgcatcgaagcgggaaggctccggcgctcggcctgagtcacctcagcagagtgatctgctgacgctcccaaccttgaataacgaaacggcaacgcctccatagcggtgcaggtcaataagggtcggccccacgcgtgtagggagcgatcgagtgacagtatcctctgtatttttatttttt

SEQ ID NO: 16 - RNA, 341 nt, synthetic construct
  source 1..341: mol_type = other RNA
gaacgcggcccggaacatcgaacgccacgcagtgctgatcgatcgaaacgtcgcctgcgataggcgggagacgctaaacgcccgtggagcatccataagaccaaccacctctcggggcggtaggcacgacgcatcgaagcgggaaggctccggcgctcggcctgagtcacctcagcagagtgatctgctgacgctcccaaccttgaataacgaaacggcaacgcctccatagcggtgcaggtcaataagggtcggccccacgcgtgtagggagcgatcgagtgacagtatcctctgtatttgacgcggttctatctagttacgcgttaaaccaactagaaa

SEQ ID NO: 17 - RNA, 349 nt, synthetic construct
  source 1..349: mol_type = other RNA
gaacgcggcccggaacatcgaacgccacgcagtgctgatcgatcgaaacgtcgcctgcgataggcgggagacgctaaacgcccgtggagcatccataagaccaaccacctctcggggcggtaggcacgacgcatcgaagcgggaaggctccggcgctcggcctgagtcacctcagcagagtgatctgctgacgctcccaaccttgaataacgaaacggcaacgcctccatagcggtgcaggtcaataagggtcggccccacgcgtgtagggagcgatcgagtgacagtatcctctgtatacatgcgattgacgcggttctatctagttacgcgttaaaccaactagaaa

SEQ ID NO: 18 - DNA, 2527 bp, synthetic construct
  source 1..2527: mol_type = other DNA
ggtgaagggggcggccgctcgaggctagtctcgtgatcgataccgtcgagatccgttcactaatcggtacctatcgatagagaaatgttctggcacctgcacttgcactggggacagcctattttgctagtttgttttgtttcgttttgttttgatggagagcgtatgttagtactatcgattcttgaccgacaattgcatgaagaatctgcttagggttaggcgttttgcgctgcttcgcgatgtacgggccagatatacgcgttgacattgattattgactagttattaatagtaatcaattacggggtcattagttcatagcccatatatggagttccgcgttacataacttacggtaaatggcccgcctggctgaccgcccaacgacccccgcccattgacgtcaataatgacgtatgttcccatagtaacgccaatagggactttccattgacgtcaatgggtggagtatttacggtaaactgcccacttggcagtacatcaagtgtatcatatgccaagtacgccccctattgacgtcaatgacggtaaatggcccgcctggcattatgcccagtacatgaccttatgggactttcctacttggcagtacatctacgtattagtcatcgctattaccatggtgatgcggttttggcagtacatcaatgggcgtggatagcggtttgactcacggggatttccaagtctccaccccattgacgtcaatgggagtttgttttggcaccaaaatcaacgggactttccaaaatgtcgtaacaactccgccccattgacgcaaatgggcggtaggcgtgtacggtgggaggtctatataagcagagctggtttagtgaaccgtcagatccgctagagatccgcggccgctaatacgactcactatagggagagccgccaccatggcccctaagaagaagaggaaggtcatggtgcagacagagatcctgaaggcctttcggttcgccctcgatcctacttccgtccaggtggccgccctgagccggcacgccggggccgccaggtgggccttcaaccacgccctcgccgccaaggtgggggcccacgagcggtggcgggccgaggtggccaagctcgtgggcgatggcgtgcccgaggagcaggcccggcggcaggtccgggtccccgtgcctatgaagccagccatccagaaggccctgaacgccgtgaagggggattcccggaagggcctggatggggcctgcccatggtggcacgaggtgaacacctacgccttccagagcgcctttattgacgccgaccaggcatggaagaactggctcgacagcctgagcggcaagagagtggggaggagggtgggctacccccggtttaagaagaagggccgggctcgggatagctttagattgcaccacgatgtgaagaagcccagcatcaggctggctggctacagaaggctgaggctgcctaggattggcgaggtgaggctgcacgacagcggcaagcggctcgccaggctcattgacagaggcgacgccgtggtgcagtccgtgactgtgagtaggggcggacacaggtggtacgcctccgtgctctgcaaggtgacagtgcaggtgcccgatcggcccagcaggcggcagcgggagaggggcgccgtgggagtggacctgggggtgaaggtgctggccgccctgtccaagcccctggtcgtcgacgacccaagcagcgccctggtgagaaacccccagcacctgaggcaggctgagaggcggctgctcaaggcccagcgggccctggccaggacacagaagggcagcgccaggagagagaaggccaagcggcgggtggggagggcccatcacgaggtggccgtccggcggcacgccgccctgcaccagatcaccaagcggctgaccacagggttcgccgtggtggccctggaggatctgaacgtcgccggcatgaccaggtccgccagggggacagtggccgccccagggaagaacgtccggcagaaggccgggctgaaccgggtcatcctggacagcgcccctgccgagctgcggaggcaggtgaactacaaggccacctggtacgggagcgagctggccgtggccgacaggtggttcccctccagcaagacctgcagcgggtgcggctggcagaacccccacttgaagctctccgatagggtgtttaggtgcaccgactgcggcctggtcatggatagagatatgaacgccgctaggaacatcgagaggcacgctgtgttgattgataggaacgtggcctgcgaccggcgggagactttgaacgccaggggggccagcatccggcccaccacaagccggggggggcggcacgacgccagcaagagggaggggagcggggcccggccagagtccccccagcagtctgatctgctcacactccccacactgaacaacgaaaccgccacacccccctctggtggttctcccaagaagaagaggaaagtctaaccggtcatcatcaccatcaccat

SEQ ID NO: 19 - DNA, 760 bp, synthetic construct
  source 1..760: mol_type = other DNA
gagggcctatttcccatgattccttcatatttgcatatacgatacaaggctgttagagagataattggaattaatttgactgtaaacacaaagatattagtacaaaatacgtgacgtagaaagtaataatttcttgggtagtttgcagttttaaaattatgttttaaaatggactatcatatgcttaccgtaacttgaaagtatttcgatttcttggctttatatatcttgtggaaaggacgaaacaccggaacgcggcccggaacatcgaacgccacgcagtgctgatcgatcgaaacgtcgcctgcgataggcgggagacgctaaacgcccgtggagcatccataagaccaaccacctctcggggcggtaggcacgacgcatcgaagcgggaaggctccggcgctcggcctgagtcacctcagcagagtgatctgctgacgctcccaaccttgaataacgaaacggcaacgcctccatagcggtgcaggtcaataagggtcggccccacgcgtgtagggagcgatcgcgagaccattggtctcatttttttgaattctcgacctcgagacaaatggcagtattcatccacaattttaaaagaaaaggggggattggggggtacagtgcaggggaaagaatagtagacataatagcaacagacatacaaactaaagaattacaaaaacaaattacaaaaattcaaaattttcgggtttattacagggacagcagagatccactttggccgcggctcgag

SEQ ID NO: 20 - DNA, 1278 bp, synthetic construct
  source 1..1278: mol_type = other DNA
ggggttggggttgcgccttttccaaggcagccctgggtttgcgcagggacgcggctgctctgggcgtggttccgggaaacgcagcggcgccgaccctgggactcgcacattcttcacgtccgttcgcagcgtcacccggatcttcgccgctacccttgtgggccccccggcgacgcttcctgctccgcccctaagtcgggaaggttccttgcggttcgcggcgtgccggacgtgacaaacggaagccgcacgtctcactagtaccctcgcagacggacagcgccagggagcaatggcagcgcgccgaccgcgatgggctgtggccaatagcggctgctcagcagggcgcgccgagagcagcggccgggaaggggcggtgcgggaggcggggtgtggggcggtagtgtgggccctgttcctgcccgcgcggtgttccgcattctgcaagcctccggagcgcacgtcggcagtcggctccctcgttgaccgaatcaccgacctctctccccagggggatccaccggagcttaccatgaccgagtacaagcccacggtgcgcctcgccacccgcgacgacgtccccagggccgtacgcaccctcgccgccgcgttcgccgactaccccgccacgcgccacaccgtcgatccggaccgccacatcgagcgggtcaccgagctgcaagaactcttcctcacgcgcgtcgggctcgacatcggcaaggtgtgggtcgcggacgacggcgccgcggtggcggtctggaccacgccggagagcgtcgaagcgggggcggtgttcgccgagatcggcccgcgcatggccgagttgagcggttcccggctggccgcgcagcaacagatggaaggcctcctggcgccgcaccggcccaaggagcccgcgtggttcctggccaccgtcggcgtctcgcccgaccaccagggcaagggtctgggcagcgccgtcgtgctccccggagtggaggcggccgagcgcgccggggtgcccgccttcctggaaacctccgcgccccgcaacctccccttctacgagcggctcggcttcaccgtcaccgccgacgtcgaggtgcccgaaggaccgcgcacctggtgcatgacccgcaagcccggtgcctgacgcccgccccacgacccgcagcgcccgaccgaaaggagcgcacgaccccatgcatcggtacctttaagaccaatgacttacaaggcagctgtagatcttagccactttctagagtcggggcggccggccgcttcgagcagacatga

SEQ ID NO: 21 - DNA, 2631 bp, synthetic construct
  source 1..2631: mol_type = other DNA
taagatacattgatgagtttggacaaaccacaactagaatgcagtgaaaaaaatgctttatttgtgaaatttgtgatgctattgctttatttgtaaccattataagctgcaataaacaagttaacaacaacaattgcattcattttatgtttcaggttcagggggaggtgtgggaggttttttaaagcaagtaaaacctctacaaatgtggtaaaatcgataaggatccgtcgaccgatgcccttgagagccttcaacccagtcagctccttccggtgggcgcggggcatgactatcgtcgccgcacttatgactgtcttctttatcatgcaactcgtaggacaggtgccggcagcgctcttccgcttcctcgctcactgactcgctgcgctcggtcgttcggctgcggcgagcggtatcagctcactcaaaggcggtaatacggttatccacagaatcaggggataacgcaggaaagaacatgtgagcaaaaggccagcaaaaggccaggaaccgtaaaaaggccgcgttgctggcgtttttccataggctccgcccccctgacgagcatcacaaaaatcgacgctcaagtcagaggtggcgaaacccgacaggactataaagataccaggcgtttccccctggaagctccctcgtgcgctctcctgttccgaccctgccgcttaccggatacctgtccgcctttctcccttcgggaagcgtggcgctttctcaatgctcacgctgtaggtatctcagttcggtgtaggtcgttcgctccaagctgggctgtgtgcacgaaccccccgttcagcccgaccgctgcgccttatccggtaactatcgtcttgagtccaacccggtaagacacgacttatcgccactggcagcagccactggtaacaggattagcagagcgaggtatgtaggcggtgctacagagttcttgaagtggtggcctaactacggctacactagaaggacagtatttggtatctgcgctctgctgaagccagttaccttcggaaaaagagttggtagctcttgatccggcaaacaaaccaccgctggtagcggtggtttttttgtttgcaagcagcagattacgcgcagaaaaaaaggatctcaagaagatcctttgatcttttctacggggtctgacgctcagtggaacgaaaactcacgttaagggattttggtcatgagattatcaaaaaggatcttcacctagatccttttaaattaaaaatgaagttttaaatcaatctaaagtatatatgagtaaacttggtctgacagttaccaatgcttaatcagtgaggcacctatctcagcgatctgtctatttcgttcatccatagttgcctgactccccgtcgtgtagataactacgatacgggagggcttaccatctggccccagtgctgcaatgataccgcgggacccacgctcaccggctccagatttatcagcaataaaccagccagccggaagggccgagcgcagaagtggtcctgcaactttatccgcctccatccagtctattaattgttgccgggaagctagagtaagtagttcgccagttaatagtttgcgcaacgttgttgccattgctacaggcatcgtggtgtcacgctcgtcgtttggtatggcttcattcagctccggttcccaacgatcaaggcgagttacatgatcccccatgttgtgcaaaaaagcggttagctccttcggtcctccgatcgttgtcagaagtaagttggccgcagtgttatcactcatggttatggcagcactgcataattctcttactgtcatgccatccgtaagatgcttttctgtgactggtgagtactcaaccaagtcattctgagaatagtgtatgcggcgaccgagttgctcttgcccggcgtcaatacgggataataccgcgccacatagcagaactttaaaagtgctcatcattggaaaacgttcttcggggcgaaaactctcaaggatcttaccgctgttgagatccagttcgatgtaacccactcgtgcacccaactgatcttcagcatcttttactttcaccagcgtttctgggtgagcaaaaacaggaaggcaaaatgccgcaaaaaagggaataagggcgacacggaaatgttgaatactcatactcttcctttttcaatattattgaagcatttatcagggttattgtctcatgagcggatacatatttgaatgtatttagaaaaataaacaaataggggttccgcgcacatttccccgaaaagtgccacctgcaggaaacagctatgaccatgattacgccaagctctagctagaggtcgacggtatcgagccccagctggttctttccgcctcagaagccatagagcccaccgcatccccagcatgcctgctattgtcttcccaatcctcccccttgctgtcctgccccaccccaccccccagaatagaatgacacctactcagacaatgcgatgcaatttcctcattttattaggaaaggacagtgggagtggcaccttccagggtcaaggaaggcacgggggaggggcaaacaacagatggctggcaactagaaggcacagtcgaggctgatcagcgggtttaaactca

SEQ ID NO: 22 - DNA, 25 bp, synthetic construct
  source 1..25: mol_type = other DNA
atcgaagtgacagtatcctctgtat

SEQ ID NO: 23 - DNA, 24 bp, synthetic construct
  source 1..24: mol_type = other DNA
aaaaatacagaggatactgtcact

SEQ ID NO: 24 - DNA, 24 bp, synthetic construct
  source 1..24: mol_type = other DNA
atcgcatggaaacagacctggcag

SEQ ID NO: 25 - DNA, 24 bp, synthetic construct
  source 1..24: mol_type = other DNA
aaaactgccaggtctgtttccatg

SEQ ID NO: 26 - DNA, 24 bp, synthetic construct
  source 1..24: mol_type = other DNA
atcgggatgtggtgcatttggaat

SEQ ID NO: 27 - DNA, 24 bp, synthetic construct
  source 1..24: mol_type = other DNA
aaaaattccaaatgcaccacatcc

SEQ ID NO: 28 - DNA, 24 bp, synthetic construct
  source 1..24: mol_type = other DNA
atcgcgactcaacctggtaaacat

SEQ ID NO: 29 - DNA, 24 bp, synthetic construct
  source 1..24: mol_type = other DNA
aaaaatgtttaccaggttgagtcg

SEQ ID NO: 30 - DNA, 24 bp, synthetic construct
  source 1..24: mol_type = other DNA
atcgaatcatttccccaagaggaa

SEQ ID NO: 31 - DNA, 24 bp, synthetic construct
  source 1..24: mol_type = other DNA
aaaattcctcttggggaaatgatt

SEQ ID NO: 32 - DNA, 24 bp, synthetic construct
  source 1..24: mol_type = other DNA
atcgaggcaagcatggaaacagac

SEQ ID NO: 33 - DNA, 24 bp, synthetic construct
  source 1..24: mol_type = other DNA
aaaagtctgtttccatgcttgcct

SEQ ID NO: 34 - DNA, 24 bp, synthetic construct
  source 1..24: mol_type = other DNA
atcgtgtttctgccaggtctgttt

SEQ ID NO: 35 - DNA, 24 bp, synthetic construct
  source 1..24: mol_type = other DNA
aaaaaaacagacctggcagaaaca

SEQ ID NO: 36 - DNA, 24 bp, synthetic construct
  source 1..24: mol_type = other DNA
atcgaagggatgtggtgcatttgg

SEQ ID NO: 37 - DNA, 24 bp, synthetic construct
  source 1..24: mol_type = other DNA
aaaaccaaatgcaccacatccctt

SEQ ID NO: 38 - DNA, 24 bp, synthetic construct
  source 1..24: mol_type = other DNA
atcgtgtaaggaagctgcagcacc

SEQ ID NO: 39 - DNA, 24 bp, synthetic construct
  source 1..24: mol_type = other DNA
aaaaggtgctgcagcttccttaca

SEQ ID NO: 40 - DNA, 24 bp, synthetic construct
  source 1..24: mol_type = other DNA
atcgggagacatccgtcggagaag

SEQ ID NO: 41 - DNA, 24 bp, synthetic construct
  source 1..24: mol_type = other DNA
aaaacttctccgacggatgtctcc

SEQ ID NO: 42 - DNA, 24 bp, synthetic construct
  source 1..24: mol_type = other DNA
atcgaaggatggagaaagagaaag

SEQ ID NO: 43 - DNA, 24 bp, synthetic construct
  source 1..24: mol_type = other DNA
aaaactttctctttctccatcctt

SEQ ID NO: 44 - DNA, 24 bp, synthetic construct
  source 1..24: mol_type = other DNA
atcgaggagaagcagtttggaaaa

SEQ ID NO: 45 - DNA, 24 bp, synthetic construct
  source 1..24: mol_type = other DNA
aaaattttccaaactgcttctcct

SEQ ID NO: 46 - DNA, 24 bp, synthetic construct
  source 1..24: mol_type = other DNA
atcgcaaaccttagaggttctggc

SEQ ID NO: 47 - DNA, 24 bp, synthetic construct
  source 1..24: mol_type = other DNA
aaaagccagaacctctaaggtttg

SEQ ID NO: 48 - DNA, 24 bp, synthetic construct
  source 1..24: mol_type = other DNA
atcggaatctgcctaacaggaggt

SEQ ID NO: 49 - DNA, 24 bp, synthetic construct
  source 1..24: mol_type = other DNA
aaaaacctcctgttaggcagattc

SEQ ID NO: 50 - DNA, 24 bp, synthetic construct
  source 1..24: mol_type = other DNA
atcggagagagatggctccaggaa

SEQ ID NO: 51 - DNA, 24 bp, synthetic construct
  source 1..24: mol_type = other DNA
aaaattcctggagccatctctctc

SEQ ID NO: 52 - DNA, 24 bp, synthetic construct
  source 1..24: mol_type = other DNA
atcgaggatggagaggtggctaaa

SEQ ID NO: 53 - DNA, 24 bp, synthetic construct
  source 1..24: mol_type = other DNA
aaaatttagccacctctccatcct

SEQ ID NO: 54 - DNA, 24 bp, synthetic construct
  source 1..24: mol_type = other DNA
atcgagctagcacagactagagag

SEQ ID NO: 55 - DNA, 24 bp, synthetic construct
  source 1..24: mol_type = other DNA
aaaactctctagtctgtgctagct

SEQ ID NO: 56 - DNA, 24 bp, synthetic construct
  source 1..24: mol_type = other DNA
atcggccatcctaagaaacgagag

SEQ ID NO: 57 - DNA, 24 bp, synthetic construct
  source 1..24: mol_type = other DNA
aaaactctcgtttcttaggatggc

SEQ ID NO: 58 - DNA, 24 bp, synthetic construct
  source 1..24: mol_type = other DNA
atcgtaccccgtctccctggcttt

SEQ ID NO: 59 - DNA, 24 bp, synthetic construct
  source 1..24: mol_type = other DNA
aaaaaaagccagggagacggggta

SEQ ID NO: 60 - DNA, 24 bp, synthetic construct
  source 1..24: mol_type = other DNA
atcgggggcaaagactggaccctg

SEQ ID NO: 61 - DNA, 24 bp, synthetic construct
  source 1..24: mol_type = other DNA
aaaacagggtccagtctttgcccc

SEQ ID NO: 62 - DNA, 24 bp, synthetic construct
  source 1..24: mol_type = other DNA
atcgctcggagctgggaccacgtg

SEQ ID NO: 63 - DNA, 24 bp, synthetic construct
  source 1..24: mol_type = other DNA
aaaacacgtggtcccagctccgag

SEQ ID NO: 64 - DNA, 24 bp, synthetic construct
  source 1..24: mol_type = other DNA
atcgacagtggggactagagctca

SEQ ID NO: 65 - DNA, 24 bp, synthetic construct
  source 1..24: mol_type = other DNA
aaaatgagctctagtccccactgt

SEQ ID NO: 66 - DNA, 24 bp, synthetic construct
  source 1..24: mol_type = other DNA
atcgcatctttgctgtgagctcta

SEQ ID NO: 67 - DNA, 24 bp, synthetic construct
  source 1..24: mol_type = other DNA
aaaatagagctcacagcaaagatg

SEQ ID NO: 68 - DNA, 24 bp, synthetic construct
  source 1..24: mol_type = other DNA
atcgatgcttcagagacgagatgg

SEQ ID NO: 69 - DNA, 24 bp, synthetic construct
  source 1..24: mol_type = other DNA
aaaaccatctcgtctctgaagcat

SEQ ID NO: 70 - DNA, 24 bp, synthetic construct
  source 1..24: mol_type = other DNA
atcggagctctacaccacacccaa

SEQ ID NO: 71 - DNA, 24 bp, synthetic construct
  source 1..24: mol_type = other DNA
aaaattgggtgtggtgtagagctc

SEQ ID NO: 72 - DNA, 24 bp, synthetic construct
  source 1..24: mol_type = other DNA
atcgcttaagcaaatgccacagct

SEQ ID NO: 73 - DNA, 24 bp, synthetic construct
  source 1..24: mol_type = other DNA
aaaaagctgtggcatttgcttaag

SEQ ID NO: 74 - DNA, 24 bp, synthetic construct
  source 1..24: mol_type = other DNA
atcgtttaactacttactgtttgt

SEQ ID NO: 75 - DNA, 24 bp, synthetic construct
  source 1..24: mol_type = other DNA
aaaaacaaacagtaagtagttaaa

SEQ ID NO: 76 - DNA, 24 bp, synthetic construct
  source 1..24: mol_type = other DNA
atcgctgtggcatttgcttaagct

SEQ ID NO: 77 - DNA, 24 bp, synthetic construct
  source 1..24: mol_type = other DNA
aaaaagcttaagcaaatgccacag

SEQ ID NO: 78 - DNA, 24 bp, synthetic construct
  source 1..24: mol_type = other DNA
atcggttgaacaaacagtaagtag

SEQ ID NO: 79 - DNA, 24 bp, synthetic construct
  source 1..24: mol_type = other DNA
aaaactacttactgtttgttcaac

SEQ ID NO: 80 - DNA, 24 bp, synthetic construct
  source 1..24: mol_type = other DNA
atcgagagatgccttactaggtac

SEQ ID NO: 81 - DNA, 24 bp, synthetic construct
  source 1..24: mol_type = other DNA
aaaagtacctagtaaggcatctct

SEQ ID NO: 82 - DNA, 24 bp, synthetic construct
  source 1..24: mol_type = other DNA
atcgagctttacaaaagaagggga

SEQ ID NO: 83 - DNA, 24 bp, synthetic construct
  source 1..24: mol_type = other DNA
aaaatccccttcttttgtaaagct

SEQ ID NO: 84 - DNA, 24 bp, synthetic construct
  source 1..24: mol_type = other DNA
atcggacaaggttgaacaaacagt

SEQ ID NO: 85 - DNA, 24 bp, synthetic construct
  source 1..24: mol_type = other DNA
aaaaactgtttgttcaaccttgtc

SEQ ID NO: 86 - DNA, 24 bp, synthetic construct
  source 1..24: mol_type = other DNA
atcgcagctcatttacagacggga

SEQ ID NO: 87 - DNA, 24 bp, synthetic construct
  source 1..24: mol_type = other DNA
aaaatcccgtctgtaaatgagctg

SEQ ID NO: 88 - DNA, 24 bp, synthetic construct
  source 1..24: mol_type = other DNA
atcggtgtcagtttaagaatggtg

SEQ ID NO: 89 - DNA, 24 bp, synthetic construct
  source 1..24: mol_type = other DNA
aaaacaccattcttaaactgacac

SEQ ID NO: 90 - DNA, 24 bp, synthetic construct
  source 1..24: mol_type = other DNA
atcgggtgcagttatgcctcagat

SEQ ID NO: 91 - DNA, 24 bp, synthetic construct
  source 1..24: mol_type = other DNA
aaaaatctgaggcataactgcacc

SEQ ID NO: 92 - DNA, 300 bp, synthetic construct
  source 1..300: mol_type = other DNA
gaacgcggcccggaacatcgaacgccacgcagtgctgatcgatcgaaacgtcgcctgcgataggcgggagacgctaaacgcccgtggagcatccataagaccaaccacctctcggggcggtaggcacgacgcatcgaagcgggaaggctccggcgctcggcctgagtcacctcagcagagtgatctgctgacgctcccaaccttgaataacgaaacggcaacgcctccatagcggtgcaggtcaataagggtcggccccacgcgtgtagggagcgatcgaagtgacagtatcctctgtat

SEQ ID NO: 93 - DNA, 241 bp, synthetic construct
  source 1..241: mol_type = other DNA
cagtgctgatcgatcgaaacgtcgcctgcgataggcgggagacgctaaacgcccgtggagcatccataagaccaaccacctctcggggcggtaggcacgacgcatcgaagcgggaaggctccggcgctcggcctgagtcacctcagcagagtgatctgctgacgctcccaaccttgaataacgaaacgaaagtcggccccacgcgtgtagggagcgatcgaagtgacagtatcctctgtat

SEQ ID NO: 94 - DNA, 232 bp, synthetic construct
  source 1..232: mol_type = other DNA
cagtgctgatcgatcgaaacgtcgcctgcgataggcgggagacgctaaacgcccgtggagcatccataagaccaaccacctctcggggcggtaggcacgacgcatcgaagcgggaaggctccggcgctcggcctgagtcacctcagcagagtgatctgctgacgctcccaaccttgaataacggaaaccccacgcgtgtagggagcgatcgaagtgacagtatcctctgtat

SEQ ID NO: 95 - DNA, 232 bp, synthetic construct; identical to SEQ ID NO: 94
  source 1..232: mol_type = other DNA

SEQ ID NO: 96 - DNA, 224 bp, synthetic construct
  source 1..224: mol_type = other DNA
cagtgctgatcgatcgaaacgtcgcctgcgataggcgggagacgctaaacgcccgtggagcatccataagaccaaccacctctcggggcggtaggcacgacgcatcgaagcgggaaggctccggcgctcggcctgagtcacctcagcagagtgatctgctgacgctcccaaccttgaatgaaaacgcgtgtagggagcgatcgaagtgacagtatcctctgtat

SEQ ID NO: 97 - DNA, 218 bp, synthetic construct
  source 1..218: mol_type = other DNA
cagtgctgatcgatcgaaacgtcgcctgcgataggcgggagacgctaaacgcccgtggagcatccataagaccaaccacctctcggggcggtaggcacgacgcatcgaagcgggaaggctccggcgctcggcctgagtcacctcagcagagtgatctgctgacgctcccaaccttggaaacgtgtagggagcgatcgaagtgacagtatcctctgtat

SEQ ID NO: 98 - DNA, 211 bp, synthetic construct
  source 1..211: mol_type = other DNA
cagtgctgatcgatcgaaacgtcgcctgcgataggcgggagacgctaaacgcccgtggagcatccataagaccaaccacctctcggggcggtaggcacgacgcatcgaagcgggaaggctccggcgctcggcctgagtcacctcagcagagtgatctgctgacgctcccaacgaaagtagggagcgatcgaagtgacagtatcctctgtat

SEQ ID NO: 99 - DNA, 205 bp, synthetic construct
  source 1..205: mol_type = other DNA
cagtgctgatcgatcgaaacgtcgcctgcgataggcgggagacgctaaacgcccgtggagcatccataagaccaaccacctctcggggcggtaggcacgacgcatcgaagcgggaaggctccggcgctcggcctgagtcacctcagcagagtgatctgctgacgctcccgaaagggagcgatcgaagtgacagtatcctctgtat

SEQ ID NO: 100 - DNA, 201 bp, synthetic construct
  source 1..201: mol_type = other DNA
cagtgctgatcgatcgaaacgtcgcctgcgataggcgggagacgctaaacgcccgtggagcatccataagaccaaccacctctcggggcggtaggcacgacgcatcgaagcgggaaggctccggcgctcggcctgagtcacctcagcagagtgatctgctgacgctcgaaagagcgatcgaagtgacagtatcctctgtat

SEQ ID NO: 101 - DNA, 197 bp, synthetic construct
  source 1..197: mol_type = other DNA
cagtgctgatcgatcgaaacgtcgcctgcgataggcgggagacgctaaacgcccgtggagcatccataagaccaaccacctctcggggcggtaggcacgacgcatcgaagcgggaaggctccggcgctcggcctgagtcacctcagcagagtgatctgctgacgcgaaagcgatcgaagtgacagtatcctctgtat

SEQ ID NO: 102 - DNA, 193 bp, synthetic construct
  source 1..193: mol_type = other DNA
cagtgctgatcgatcgaaacgtcgcctgcgataggcgggagacgctaaacgcccgtggagcatccataagaccaaccacctctcggggcggtaggcacgacgcatcgaagcgggaaggctccggcgctcggcctgagtcacctcagcagagtgatctgctgacgaaagatcgaagtgacagtatcctctgtat

SEQ ID NO: 103 - DNA, 311 bp, synthetic construct
  source 1..311: mol_type = other DNA
gaacgcggcccggaacatcgaacgccacgcagtgctgatcgatcgaaacgtcgcctgcgataggcgggagacgctaaacgcccgtggagcatccataagaccaaccacctctcggggcggtaggcacgacgcatcgaagcgggaaggctccggcgctcggcctgagtcacctcagcagagtgatctgctgacgctcccaaccttgaataacgaaacggcaacgcctccatagcggtgcaggtcaataagggtcggccccacgcgtgtagggagcgatcgaagtgacagtatcctctgtatttttatttttt

SEQ ID NO: 104 - DNA, 342 bp, synthetic construct
  source 1..342: mol_type = other DNA
gaacgcggcccggaacatcgaacgccacgcagtgctgatcgatcgaaacgtcgcctgcgataggcgggagacgctaaacgcccgtggagcatccataagaccaaccacctctcggggcggtaggcacgacgcatcgaagcgggaaggctccggcgctcggcctgagtcacctcagcagagtgatctgctgacgctcccaaccttgaataacgaaacggcaacgcctccatagcggtgcaggtcaataagggtcggccccacgcgtgtagggagcgatcgaagtgacagtatcctctgtatttgacgcggttctatctagttacgcgttaaaccaactagaaa

SEQ ID NO: 105 - DNA, 350 bp, synthetic construct
  source 1..350: mol_type = other DNA
gaacgcggcccggaacatcgaacgccacgcagtgctgatcgatcgaaacgtcgcctgcgataggcgggagacgctaaacgcccgtggagcatccataagaccaaccacctctcggggcggtaggcacgacgcatcgaagcgggaaggctccggcgctcggcctgagtcacctcagcagagtgatctgctgacgctcccaaccttgaataacgaaacggcaacgcctccatagcggtgcaggtcaataagggtcggccccacgcgtgtagggagcgatcgaagtgacagtatcctctgtatacatgcgattgacgcggttctatctagttacgcgttaaaccaactagaaa

SEQ ID NO: 106 - RNA, 279 nt, synthetic construct
  source 1..279: mol_type = other RNA
gaacgcggcccggaacatcgaacgccacgcagtgctgatcgatcgaaacgtcgcctgcgataggcgggagacgctaaacgcccgtggagcatccataagaccaaccacctctcggggcggtaggcacgacgcatcgaagcgggaaggctccggcgctcggcctgagtcacctcagcagagtgatctgctgacgctcccaaccttgaataacgaaacggcaacgcctccatagcggtgcaggtcaataagggtcggccccacgcgtgtagggagcgatcg

SEQ ID NO: 107 - RNA, 250 nt, synthetic construct
  source 1..250: mol_type = other RNA
cagtgctgatcgatcgaaacgtcgcctgcgataggcgggagacgctaaacgcccgtggagcatccataagaccaaccacctctcggggcggtaggcacgacgcatcgaagcgggaaggctccggcgctcggcctgagtcacctcagcagagtgatctgctgacgctcccaaccttgaataacgaaacggcaacgcctccatagcggtgcaggtcaataagggtcggccccacgcgtgtagggagcgatcg

SEQ ID NO: 108 - RNA, 220 nt, synthetic construct
  source 1..220: mol_type = other RNA
cagtgctgatcgatcgaaacgtcgcctgcgataggcgggagacgctaaacgcccgtggagcatccataagaccaaccacctctcggggcggtaggcacgacgcatcgaagcgggaaggctccggcgctcggcctgagtcacctcagcagagtgatctgctgacgctcccaaccttgaataacgaaacgaaagtcggccccacgcgtgtagggagcgatcg

SEQ ID NO: 109 - RNA, 211 nt, synthetic construct
  source 1..211: mol_type = other RNA
cagtgctgatcgatcgaaacgtcgcctgcgataggcgggagacgctaaacgcccgtggagcatccataagaccaaccacctctcggggcggtaggcacgacgcatcgaagcgggaaggctccggcgctcggcctgagtcacctcagcagagtgatctgctgacgctcccaaccttgaataacggaaaccccacgcgtgtagggagcgatcg

SEQ ID NO: 110 - RNA, 203 nt, synthetic construct
  source 1..203: mol_type = other RNA
cagtgctgatcgatcgaaacgtcgcctgcgataggcgggagacgctaaacgcccgtggagcatccataagaccaaccacctctcggggcggtaggcacgacgcatcgaagcgggaaggctccggcgctcggcctgagtcacctcagcagagtgatctgctgacgctcccaaccttgaatgaaaacgcgtgtagggagcgatcg

SEQ ID NO: 111 - RNA, 197 nt, synthetic construct
  source 1..197: mol_type = other RNA
cagtgctgatcgatcgaaacgtcgcctgcgataggcgggagacgctaaacgcccgtggagcatccataagaccaaccacctctcggggcggtaggcacgacgcatcgaagcgggaaggctccggcgctcggcctgagtcacctcagcagagtgatctgctgacgctcccaaccttggaaacgtgtagggagcgatcg

SEQ ID NO: 112 - RNA, 190 nt, synthetic construct
  source 1..190: mol_type = other RNA
cagtgctgatcgatcgaaacgtcgcctgcgataggcgggagacgctaaacgcccgtggagcatccataagaccaaccacctctcggggcggtaggcacgacgcatcgaagcgggaaggctccggcgctcggcctgagtcacctcagcagagtgatctgctgacgctcccaacgaaagtagggagcgatcg

SEQ ID NO: 113 - RNA, 184 nt, synthetic construct
  source 1..184: mol_type = other RNA
cagtgctgatcgatcgaaacgtcgcctgcgataggcgggagacgctaaacgcccgtggagcatccataagaccaaccacctctcggggcggtaggcacgacgcatcgaagcgggaaggctccggcgctcggcctgagtcacctcagcagagtgatctgctgacgctcccgaaagggagcgatcg

SEQ ID NO: 114 - RNA, 180 nt, synthetic construct
  source 1..180: mol_type = other RNA
cagtgctgatcgatcgaaacgtcgcctgcgataggcgggagacgctaaacgcccgtggagcatccataagaccaaccacctctcggggcggtaggcacgacgcatcgaagcgggaaggctccggcgctcggcctgagtcacctcagcagagtgatctgctgacgctcgaaagagcgatcg

SEQ ID NO: 115 - RNA, 176 nt, synthetic construct
  source 1..176: mol_type = other RNA
cagtgctgatcgatcgaaacgtcgcctgcgataggcgggagacgctaaacgcccgtggagcatccataagaccaaccacctctcggggcggtaggcacgacgcatcgaagcgggaaggctccggcgctcggcctgagtcacctcagcagagtgatctgctgacgcgaaagcgatcg

SEQ ID NO: 116 - RNA, 172 nt, synthetic construct
  source 1..172: mol_type = other RNA
cagtgctgatcgatcgaaacgtcgcctgcgataggcgggagacgctaaacgcccgtggagcatccataagaccaaccacctctcggggcggtaggcacgacgcatcgaagcgggaaggctccggcgctcggcctgagtcacctcagcagagtgatctgctgacgaaagatcg

SEQ ID NO: 117 - RNA, 224 nt, synthetic construct
  source 1..224: mol_type = other RNA
gaacgcggcccggaacatcgaacgccacgcagtgctgatcgatcgaaacgtcgcctgcgataggcgggagacgctaaacgcccgtggagcatccataagaccaaccacctctcggggcggtaggcacgacgcatcgaagcgggaaggctccggcgctcggcctgagtcacctcagcagagtgatctgctgacgctcccaaccttgaataacgaaacggcaacgc

SEQ ID NO: 118 - RNA, 187 nt, synthetic construct
  source 1..187: mol_type = other RNA
cagtgctgatcgatcgaaacgtcgcctgcgataggcgggagacgctaaacgcccgtggagcatccataagaccaaccacctctcggggcggtaggcacgacgcatcgaagcgggaaggctccggcgctcggcctgagtcacctcagcagagtgatctgctgacgctcccaaccttgaataacgaaac

SEQ ID NO: 119 - RNA, 183 nt, synthetic construct
  source 1..183: mol_type = other RNA
cagtgctgatcgatcgaaacgtcgcctgcgataggcgggagacgctaaacgcccgtggagcatccataagaccaaccacctctcggggcggtaggcacgacgcatcgaagcgggaaggctccggcgctcggcctgagtcacctcagcagagtgatctgctgacgctcccaaccttgaataacg

SEQ ID NO: 120 - RNA, 179 nt, synthetic construct
  source 1..179: mol_type = other RNA
cagtgctgatcgatcgaaacgtcgcctgcgataggcgggagacgctaaacgcccgtggagcatccataagaccaaccacctctcggggcggtaggcacgacgcatcgaagcgggaaggctccggcgctcggcctgagtcacctcagcagagtgatctgctgacgctcccaaccttgaat

SEQ ID NO: 121 - RNA, 176 nt, synthetic construct
  source 1..176: mol_type = other RNA
cagtgctgatcgatcgaaacgtcgcctgcgataggcgggagacgctaaacgcccgtggagcatccataagaccaaccacctctcggggcggtaggcacgacgcatcgaagcgggaaggctccggcgctcggcctgagtcacctcagcagagtgatctgctgacgctcccaaccttg

SEQ ID NO: 122 - RNA, 172 nt, synthetic construct
  source 1..172: mol_type = other RNA
cagtgctgatcgatcgaaacgtcgcctgcgataggcgggagacgctaaacgcccgtggagcatccataagaccaaccacctctcggggcggtaggcacgacgcatcgaagcgggaaggctccggcgctcggcctgagtcacctcagcagagtgatctgctgacgctcccaac

SEQ ID NO: 123 - RNA, 169 nt, synthetic construct
  source 1..169: mol_type = other RNA
cagtgctgatcgatcgaaacgtcgcctgcgataggcgggagacgctaaacgcccgtggagcatccataagaccaaccacctctcggggcggtaggcacgacgcatcgaagcgggaaggctccggcgctcggcctgagtcacctcagcagagtgatctgctgacgctccc

SEQ ID NO: 124 - RNA, 167 nt, synthetic construct
  source 1..167: mol_type = other RNA
cagtgctgatcgatcgaaacgtcgcctgcgataggcgggagacgctaaacgcccgtggagcatccataagaccaaccacctctcggggcggtaggcacgacgcatcgaagcgggaaggctccggcgctcggcctgagtcacctcagcagagtgatctgctgacgctc

SEQ ID NO: 125 - RNA, 165 nt, synthetic construct
  source 1..165: mol_type = other RNA
cagtgctgatcgatcgaaacgtcgcctgcgataggcgggagacgctaaacgcccgtggagcatccataagaccaaccacctctcggggcggtaggcacgacgcatcgaagcgggaaggctccggcgctcggcctgagtcacctcagcagagtgatctgctgacgc

SEQ ID NO: 126 - RNA, 163 nt, synthetic construct
  source 1..163: mol_type = other RNA
cagtgctgatcgatcgaaacgtcgcctgcgataggcgggagacgctaaacgcccgtggagcatccataagaccaaccacctctcggggcggtaggcacgacgcatcgaagcgggaaggctccggcgctcggcctgagtcacctcagcagagtgatctgctgac

SEQ ID NO: 127 - RNA, 44 nt, synthetic construct
  source 1..44: mol_type = other RNA
gcggtgcaggtcaataagggtcggccccacgcgtgtagggagcg

SEQ ID NO: 128 - RNA, 25 nt, synthetic construct
  source 1..25: mol_type = other RNA
gtcggccccacgcgtgtagggagcg

SEQ ID NO: 129 - RNA, 20 nt, synthetic construct
  source 1..20: mol_type = other RNA
ccccacgcgtgtagggagcg

SEQ ID NO: 130 - RNA, 16 nt, synthetic construct
  source 1..16: mol_type = other RNA
acgcgtgtagggagcg

SEQ ID NO: 131 - RNA, 13 nt, synthetic construct
  source 1..13: mol_type = other RNA
cgtgtagggagcg

SEQ ID NO: 132 - RNA, 10 nt, synthetic construct
  source 1..10: mol_type = other RNA
gtagggagcg

SEQ ID NO: 133-136 - skipped (4 entries)

SEQ ID NO: 137 - RNA, 11 nt, synthetic construct
  source 1..11: mol_type = other RNA
ttttatttttt

SEQ ID NO: 138 - RNA, 42 nt, synthetic construct
  source 1..42: mol_type = other RNA
ttgacgcggttctatctagttacgcgttaaaccaactagaaa

SEQ ID NO: 139 - RNA, 50 nt, synthetic construct
  source 1..50: mol_type = other RNA
acatgcgattgacgcggttctatctagttacgcgttaaaccaactagaaa

SEQ ID NO: 140 - RNA, 195 nt, synthetic construct
  source 1..195: mol_type = other RNA
cagtgctgatcgatcgaaacgtcgcctgcgataggcgggagacgctaaacgcccgtggagcatccataagaccaaccacctctcggggcggtaggcacgacgcatcgaagcgggaaggctccggcgctcggcctgagtcacctcagcagagtgatctgctgacgctcccaaccttgaataacgaaacggcaacgc